European Patent Application EP 4 446 434 A1, published October 16, 2024. Title: Method of detecting mutants in a sequence of interest, mehod of inhibiting nucleic acid amplification, kit for carrying out the methods, and agent for enhancing amplification inhibitory effect. Applicant: 日東紡績株式会社. The sequence listing filed with the application follows.

SEQUENCE LISTING (13 sequences)

SEQ ID NO: 1 - DNA, 24 bp, synthetic construct
  misc_feature 1..24: note = Forward primer
  source 1..24: mol_type = other DNA
gcctgctgaaaatgactgaatata

SEQ ID NO: 2 - DNA, 23 bp, synthetic construct
  misc_feature 1..23: note = Reverse primer
  source 1..23: mol_type = other DNA
caagatttacctctattgttgga

SEQ ID NO: 3 - DNA, 132 bp, HCC70 strain genome
  misc_feature 1..132: note = Template DNA
  source 1..132: mol_type = genomic DNA
gcctgctgaaaatgactgaatataaacttgtggtagttggagctggtggcgtaggcaagagtgccttgacgatacagctaattcagaatcattttgtggacgaatatgatccaacaatagaggtaaatcttg

SEQ ID NO: 4 - DNA, 300 bp, HCC70 strain genome
  source 1..300: mol_type = genomic DNA
tgagtttgtattaaaaggtactggtggagtatttgatagtgtattaaccttatgtgtgacatgttctaatatagtcacattttcattatttttattataaggcctgctgaaaatgactgaatataaacttgtggtagttggagctggtggcgtaggcaagagtgccttgacgatacagctaattcagaatcattttgtggacgaatatgatccaacaatagaggtaaatcttgttttaatatgcatattactggtgcaggaccattctttgatacacgataaaggtttctctgaccattt

SEQ ID NO: 5 - DNA, 25 bp, synthetic construct
  misc_feature 1..25: note = Forward primer
  source 1..25: mol_type = other DNA
ctgaatataaacttgtggtagttgg

SEQ ID NO: 6 - DNA, 20 bp, synthetic construct
  misc_feature 1..20: note = Reverse primer
  source 1..20: mol_type = other DNA
gtcctgcaccagtaatatgc

SEQ ID NO: 7 - DNA, 11 bp, synthetic construct
  misc_feature 1..2: note = 2',4'-BNANC(N-H)-cytosine
  misc_feature 3: note = 2',4'-BNANC(N-H)-thymine
  misc_feature 5: note = 2',4'-BNANC(N-H)-cytosine
  misc_feature 7..8: note = 2',4'-BNANC(N-H)-cytosine
  misc_feature 10..11: note = 2',4'-BNANC(N-H)-cytosine
  source 1..11: mol_type = other DNA
cctacgccacc

SEQ ID NO: 8 - DNA, 146 bp, HCC70 strain genome
  misc_feature 1..146: note = Template DNA
  source 1..146: mol_type = genomic DNA
ctgaatataaacttgtggtagttggagctggtggcgtaggcaagagtgccttgacgatacagctaattcagaatcattttgtggacgaatatgatccaacaatagaggtaaatcttgttttaatatgcatattactggtgcaggac

SEQ ID NO: 9 - DNA, 300 bp, HCC70 strain genome; identical to SEQ ID NO: 4
  source 1..300: mol_type = genomic DNA

SEQ ID NO: 10 - DNA, 146 bp, MDA-MB-231 strain genome
  misc_feature 1..146: note = Template DNA
  source 1..146: mol_type = genomic DNA
ctgaatataaacttgtggtagttggagctggtgacgtaggcaagagtgccttgacgatacagctaattcagaatcattttgtggacgaatatgatccaacaatagaggtaaatcttgttttaatatgcatattactggtgcaggac

SEQ ID NO: 11 - DNA, 300 bp, MDA-MB-231 strain genome
  source 1..300: mol_type = genomic DNA
tgagtttgtattaaaaggtactggtggagtatttgatagtgtattaaccttatgtgtgacatgttctaatatagtcacattttcattatttttattataaggcctgctgaaaatgactgaatataaacttgtggtagttggagctggtgacgtaggcaagagtgccttgacgatacagctaattcagaatcattttgtggacgaatatgatccaacaatagaggtaaatcttgttttaatatgcatattactggtgcaggaccattctttgatacacgataaaggtttctctgaccattt

SEQ ID NO: 12 - DNA, 300 bp, HCC70 strain genome
  source 1..300: mol_type = genomic DNA
atagaaattagatctcttacctaaactcttcataatgcttgctctgataggaaaatgagatctactgttttcctttacttactacacctcagatatatttcttcatgaagacctcacagtaaaaataggtgattttggtctagctacagtgaaatctcgatggagtgggtcccatcagtttgaacagttgtctggatccattttgtggatggtaagaattgaggctatttttccactgattaaatttttggccctgagatgctgctgagttactagaaagtcattgaaggtctcaactat

SEQ ID NO: 13 - DNA, 300 bp, DU4475 strain genome
  source 1..300: mol_type = genomic DNA
atagaaattagatctcttacctaaactcttcataatgcttgctctgataggaaaatgagatctactgttttcctttacttactacacctcagatatatttcttcatgaagacctcacagtaaaaataggtgattttggtctagctacagagaaatctcgatggagtgggtcccatcagtttgaacagttgtctggatccattttgtggatggtaagaattgaggctatttttccactgattaaatttttggccctgagatgctgctgagttactagaaagtcattgaaggtctcaactat